European Patent Specification EP 3 947 418 B1, published April 3, 2024. Title: Peptides and Use Thereof. Applicant: Warenius, Hilmar M. The sequence listing filed with the application follows.

SEQUENCE LISTING (23 sequences)

SEQ ID NO: 1 - protein, 6 aa, Artificial Sequence
  CDK4 fragment
PRGPRP

SEQ ID NO: 2 - protein, 17 aa, Artificial Sequence
  HILR-001
PRGPRPVALKLALKLAL

SEQ ID NO: 3 - protein, 17 aa, Artificial Sequence
  HILR-PRO-25
PRGPRPVWWRRWWRRWW

SEQ ID NO: 4 - protein, 6 aa, Artificial Sequence
  Active region of peptide
  Dac (1)..(1): Dac = amino acid residue of (7-methoxy-coumarin-4-yl)-Ala-OH
  Sar (3)..(3): Sar = Sarcosine
  dmPro (4)..(4): dmPro = 5, 5-dimethylproline
  Nap (6)..(6): Nap = amino acid residue of 3-amino-3-(2-naphthyl)propionic acid
XRXXRX

SEQ ID NO: 5 - protein, 6 aa, Artificial Sequence
  Alternative active region of peptide
  Dac (1)..(1): Dac = amino acid residue of (7-methoxy-coumarin-4-yl)-Ala-OH
  Sar (3)..(3): Sar = Sarcosine
  Nap (4)..(4): Nap = amino acid residue of 3-amino-3-(2-naphthyl)propionic acid
  Nap (6)..(6): Nap = amino acid residue of 3-amino-3-(2-naphthyl)propionic acid
XRXXRX

SEQ ID NO: 6 - protein, 8 aa, Artificial Sequence
  SEQ ID NO:6
  Dac (2)..(2): Dac = amino acid residue of (7-methoxy-coumarin-4-yl)-Ala-OH
  Sar (4)..(4): Sar = Sarcosine
  dmPro (5)..(5): dmPro = 5, 5-dimethylproline dmPro can be either (S) or (R) stereoisomer
  Nap (7)..(7): Nap = amino acid residue of 3-amino-3-(2-naphthyl)propionic acid Nap can be either (S) or (R) stereoisomer
CXRXXRXC

SEQ ID NO: 7 - protein, 8 aa, Artificial Sequence
  SEQ ID NO:7
  Dac (2)..(2): Dac = amino acid residue of (7-methoxy-coumarin-4-yl)-Ala-OH
  Sar (4)..(4): Sar = Sarcosine
  Nap (5)..(5): Nap = amino acid residue of 3-amino-3-(2-naphthyl)propionic acid Nap can be (S) or (R) stereoisomer
  Nap (7)..(7): Nap = amino acid residue of 3-amino-3-(2-naphthyl)propionic acid Nap can be (S) or (R) stereoisomer
CXRXXRXC

SEQ ID NO: 8 - protein, 8 aa, Artificial Sequence
  HILRa-CL-01
CPRGPRPC

SEQ ID NO: 9 - protein, 10 aa, Artificial Sequence
  HILRa-CL-02
  Sar (2)..(2): X = Sarcosine
  Sar (9)..(9): X = Sarcosine
CXPRGPRPXC

SEQ ID NO: 10 - protein, 12 aa, Artificial Sequence
  HILRa-CL-03
  Sar (2)..(2): X = Sarcosine
  Sar (3)..(3): X = Sarcosine
  Sar (10)..(10): X = Sarcosine
  Sar (11)..(11): X = Sarcosine
CXXPRGPRPXXC

SEQ ID NO: 11 - protein, 8 aa, Artificial Sequence
  HILRa-CL-04
CPKGPRPC

SEQ ID NO: 12 - protein, 10 aa, Artificial Sequence
  HILRa-CL-05
  Sar (2)..(2): X = Sarcosine
  Sar (9)..(9): X = Sarcosine
CXPKGPRPXC

SEQ ID NO: 13 - protein, 12 aa, Artificial Sequence
  HILRa-CL-06
  Sar (2)..(2): X = Sarcosine
  Sar (3)..(3): X = Sarcosine
  Sar (10)..(10): X = Sarcosine
  Sar (11)..(11): X = Sarcosine
CXXPKGPRPXXC

SEQ ID NO: 14 - protein, 8 aa, Artificial Sequence
  HILRa-CL-07
CPRGPKPC

SEQ ID NO: 15 - protein, 10 aa, Artificial Sequence
  HILRa-CL-08
  Sar (2)..(2): X = Sarcosine
  Sar (9)..(9): X = Sarcosine
CXPRGPKPXC

SEQ ID NO: 16 - protein, 12 aa, Artificial Sequence
  HILRa-CL-9
  Sar (2)..(2): X = Sarcosine
  Sar (3)..(3): X = Sarcosine
  Sar (10)..(10): X = Sarcosine
  Sar (11)..(11): X = Sarcosine
CXXPRGPKPXXC

SEQ ID NO: 17 - protein, 8 aa, Artificial Sequence
  HILRa-CL-10
CPKGPKPC

SEQ ID NO: 18 - protein, 10 aa, Artificial Sequence
  HILRa-CL-11
  Sar (2)..(2): X = Sarcosine
  Sar (9)..(9): X = Sarcosine
CXPKGPKPXC

SEQ ID NO: 19 - protein, 12 aa, Artificial Sequence
  HILRa-CL-12
  Sar (2)..(2): X = Sarcosine
  Sar (3)..(3): X = Sarcosine
  Sar (10)..(10): X = Sarcosine
  Sar (11)..(11): X = Sarcosine
CXXPKGPKPXXC

SEQ ID NO: 20 - protein, 8 aa, Artificial Sequence
  HILRa CL-14
  Dac (2)..(2): Dac = amino acid residue of (7-methoxy-coumarin-4-yl)-Ala-OH
  Hca (3)..(3): Hca = amino acid residue of homocysteic acid
  Sar (4)..(4): Sar = Sarcosine
  Hca (6)..(6): Hca = amino acid residue of homocysteic acid
  Nap (7)..(7): Nap = amino acid residue of 3-amino-3-(2-naphthyl)propionic acid
CXXXPXXC

SEQ ID NO: 21 - protein, 8 aa, Artificial Sequence
  HILRa CL-16
  Dac (2)..(2): Dac = amino acid residue of (7-methoxy-coumarin-4-yl)-Ala-OH
  Hca (3)..(3): Hca = amino acid residue of homocysteic acid
  Sar (4)..(4): Sar = Sarcosine
  Nap (5)..(5): Nap = amino acid residue of 3-amino-3-(2-naphthyl)propionic acid
  Hca (6)..(6): Hca = amino acid residue of homocysteic acid
  Nap (7)..(7): Nap = amino acid residue of 3-amino-3-(2-naphthyl)propionic acid
CXXXXXXC

SEQ ID NO: 22 - protein, 18 aa, Artificial Sequence
  DAC peptide
  Dac (7)..(7): Dac - amino acid residue of (7-methoxy-coumarin-4-yl)-Ala-OH
  misc_feature (8)..(8): Xaa can be any naturally occurring amino acid
CPRGPRPXWWRRWWRRWW

SEQ ID NO: 23 - protein, 15 aa, Artificial Sequence
  Hilra-025
PRGPRPVWWRRWWRR